European Patent Application EP 4 177 343 A1, published May 10, 2023. Title: METHOD FOR ACTIVATING EXPRESSION OF GAMMA-GLOBIN GENE, AND COMPOSITION. Applicant: GUANGZHOU REFORGENE MEDICINE CO., LTD. Application 20942540.4. The sequence listing filed with the application follows.

SEQUENCE LISTING (79 sequences)

SEQ ID NO: 1 - DNA, 1500 bp, Homo sapiens
tctttctggccttttagccatctgtatcaatgagcagatataagctttacacaggatcatgaaggatgaaagaatttcaccaatattataataatttcaatcaacctgatagcttaggggataaactaatttgaagatacagcttgcctccgataagccagaattccagagcttctggcattataatctagcaaggttagagatcatggatcactttcagagaaaaacaaaaacaaactaaccaaaagcaaaacagaaccaaaaaaccaccataaatacttcctaccctgttaatggtccaatatgtcagaaacagcactgtgttagaaataaagctgtctaaagtacactaatattcgagttataatagtgtgtggactattagtcaataaaaacaacccttgcctctttagagttgttttccatgtacacgcacatcttatgtcttagagtaagattccctgagaagtgaacctagcatttatacaagataattaattctaatccacagtacctgccaaagaacattctaccatcatctttactgagcatagaagagctacgccaaaaccctgggtcatcagccagcacacacacttatccagtggtaaatacacatcatctggtgtatacatacatacctgaatatggaatcaaatatttttctaagatgaaacagtcatgatttatttcaaataggtacggataagtagatattgaggtaagcattaggtcttatattatgtaacactaatctattactgcgctgaaactgtggctttatagaaattgttttcactgcactattgagaaattaagagataatggcaaaagtcacaaagagtatattcaaaaagaagtatagcactttttccttagaaaccactgctaactgaaagagactaagatttgtcccgtcaaaaatcctggacctatgcctaaaacacatttcacaatccctgaacttttcaaaaattggtacatgctttagctttaaactacaggcctcactggagctagagacaagaaggtaaaaaacggctgacaaaagaagtcctggtatcctctatgatgggagaaggaaactagctaaagggaagaataaattagagaaaaactggaatgactgaatcggaacaaggcaaaggctataaaaaaaattagcagtatcctcttgggggccccttccccacactatctcaatgcaaatatctgtctgaaacggtccctggctaaactccacccatgggttggccagccttgccttgaccaatagccttgacaaggcaaacttgaccaatagtcttagagtatccagtgaggccaggggccggcggctggctagggatgaagaataaaaggaagcacccttcagcagttccacacactcgcttctggaacgtctgaggttatcaataagctcctagtccagacgccatgggtcatttcacagaggaggacaaggctactatcacaagcctgtggggcaaggtgaatgtg

SEQ ID NO: 2 - DNA, 1500 bp, Homo sapiens
atctttctggtcttttagccgcctaacactttgagcagatataagccttacacaggattatgaagtctgaaaggattccaccaatattattataattcctatcaacctgataggttaggggaaggtagagctctcctccaataagccagatttccagagtttctgacgtcataatctaccaaggtcatggatcgagttcagagaaaaaacaaaagcaaaaccaaacctaccaaaaaataaaaatcccaaagaaaaaataaagaaaaaaacagcatgaatacttcctgccatgttaagtggccaatatgtcagaaacagcactgagttacagataaagatgtctaaactacagtgacatcccagctgtcacagtgtgtggactattagtcaataaaacagtccctgcctcttaagagttgttttccatgcaaatacatgtcttatgtcttagaataagattccctaagaagtgaacctagcatttatacaagataattaattctaatccatagtatctggtaaagagcattctaccatcatctttaccgagcatagaagagctacaccaaaaccctgggtcatcagccagcacatacacttatccagtgataaatacacatcatcgggtgcctacatacatacctgaatataaaaaaaatacttttgctgagatgaaacaggcgtgatttatttcaaataggtacggataagtagatattgaagtaaggattcagtcttatattatattacataacattaatctattcctgcactgaaactgttgctttataggatttttcactacactaatgagaacttaagagataatggcctaaaaccacagagagtatattcaaagataagtatagcacttcttatttggaaaccaatgcttactaaatgagactaagacgtgtcccatcaaaaatcctggacctatgcctaaaacacatttcacaatccctgaacttttcaaaaattggtacatgctttaactttaaactacaggcctcactggagctacagacaagaaggtgaaaaacggctgacaaaagaagtcctggtatcttctatggtgggagaagaaaactagctaaagggaagaataaattagagaaaaattggaatgactgaatcggaacaaggcaaaggctataaaaaaaattaagcagcagtatcctcttgggggccccttccccacactatctcaatgcaaatatctgtctgaaacggtccctggctaaactccacccatgggttggccagccttgccttgaccaatagccttgacaaggcaaacttgaccaatagtcttagagtatccagtgaggccaggggccggcggctggctagggatgaagaataaaaggaagcacccttcagcagttccacacactcgcttctggaacgtctgaggttatcaataagctcctagtccagacgccatgggtcatttcacagaggaggacaaggctactatcacaagcctgtggggcaagg

SEQ ID NO: 3 - DNA, 27 bp, Homo sapiens
ttgaccaatagtcttagagtatccagt

SEQ ID NO: 4 - DNA, 27 bp, Artificial Sequence
  Mutant_01
ttgaccaatagtgatagagtatccagt

SEQ ID NO: 5 - DNA, 27 bp, Artificial Sequence
  Mutant_02
ttgaccaatagagatagagtatccagt

SEQ ID NO: 6 - DNA, 26 bp, Artificial Sequence
  Mutant_03
ttgaccaataagatagagtatccagt

SEQ ID NO: 7 - DNA, 26 bp, Artificial Sequence
  Mutant_04
ttgaccaatatgatagagtatccagt

SEQ ID NO: 8 - DNA, 32 bp, Homo sapiens
cagccttgccttgaccaatagccttgacaagg

SEQ ID NO: 9 - DNA, 32 bp, Artificial Sequence
  Mutant_05
cagccttgccttgacagatagccttgacaagg

SEQ ID NO: 10 - DNA, 32 bp, Artificial Sequence
  Mutant_06
cagccttgccttgactgatagccttgacaagg

SEQ ID NO: 11 - DNA, 32 bp, Artificial Sequence
  Mutant_07
cagccttgccttgagagatagccttgacaagg

SEQ ID NO: 12 - DNA, 32 bp, Artificial Sequence
  Mutant_08
cagccttgccttgagtgatagccttgacaagg

SEQ ID NO: 13 - DNA, 32 bp, Artificial Sequence
  Mutant_09
cagccttgccttgaaagatagccttgacaagg

SEQ ID NO: 14 - DNA, 32 bp, Artificial Sequence
  Mutant_10
cagccttgccttgaatgatagccttgacaagg

SEQ ID NO: 15 - DNA, 32 bp, Artificial Sequence
  Mutant_11
cagccttgccttgatagatagccttgacaagg

SEQ ID NO: 16 - DNA, 32 bp, Artificial Sequence
  Mutant_12
cagccttgccttgattgatagccttgacaagg

SEQ ID NO: 17 - DNA, 32 bp, Artificial Sequence
  Mutant_13
cagccttgccttgataaatagccttgacaagg

SEQ ID NO: 18 - DNA, 33 bp, Artificial Sequence
  Mutant_14
cagccttgccttgataaaatagccttgacaagg

SEQ ID NO: 19 - DNA, 31 bp, Artificial Sequence
  Mutant_15
cagccttgccttgataatagccttgacaagg

SEQ ID NO: 20 - DNA, 28 bp, Artificial Sequence
  Mutant_16
cagccttgccttgatagccttgacaagg

SEQ ID NO: 21 - DNA, 19 bp, Artificial Sequence
  Mutant_17
cagccttgccttgataagg

SEQ ID NO: 22 - DNA, 20 bp, Artificial Sequence
  Mutant_18
cagccttgccttgataaagg

SEQ ID NO: 23 - DNA, 23 bp, Homo sapiens
tatctgtctgaaacggtccctgg

SEQ ID NO: 24 - DNA, 29 bp, Artificial Sequence
  Mutant_19
tatctgtctgaaacggtagataaccctgg

SEQ ID NO: 25 - DNA, 33 bp, Homo sapiens
cactatctcaatgcaaatatctgtctgaaacgg

SEQ ID NO: 26 - DNA, 25 bp, Artificial Sequence
  Mutant_20
cactatctcaatgcaacagaaacgg

SEQ ID NO: 27 - DNA, 23 bp, Homo sapiens
tccctgaacttttcaaaaattgg

SEQ ID NO: 28 - DNA, 24 bp, Artificial Sequence
  Mutant_21
tccctgaacttttcagataattgg

SEQ ID NO: 29 - DNA, 25 bp, Artificial Sequence
  Mutant_22
tccctgaacttttcagataaattgg

SEQ ID NO: 30 - DNA, 26 bp, Artificial Sequence
  Mutant_23
tccctgaacttttcagataaaattgg

SEQ ID NO: 31 - DNA, 26 bp, Artificial Sequence
  Mutant_24
tccctgaacttttcagatagaattgg

SEQ ID NO: 32 - DNA, 23 bp, Homo sapiens
actggatactctaagactattgg

SEQ ID NO: 33 - DNA, 23 bp, Homo sapiens
cttgtcaaggctattggtcaagg

SEQ ID NO: 34 - DNA, 23 bp, Homo sapiens
gtttgccttgtcaaggctattgg

SEQ ID NO: 35 - DNA, 23 bp, Homo sapiens
tggtcaagtttgccttgtcaagg

SEQ ID NO: 36 - DNA, 23 bp, Homo sapiens
cttgaccaatagccttgacaagg

SEQ ID NO: 37 - DNA, 23 bp, Homo sapiens
tatctgtctgaaacggtccctgg

SEQ ID NO: 38 - DNA, 23 bp, Homo sapiens
atgcaaatatctgtctgaaacgg

SEQ ID NO: 39 - DNA, 23 bp, Homo sapiens
tccctgaacttttcaaaaattgg

SEQ ID NO: 40 - DNA, 84 bp, Artificial Sequence
  ssODN_1
cctagccagccgccggcccctggcctcactggatactctatcactattggtcaagtttgccttgtcaaggctattggtcaaggc

SEQ ID NO: 41 - DNA, 84 bp, Artificial Sequence
  ssODN_2
cctagccagccgccggcccctggcctcactggatactctatctctattggtcaagtttgccttgtcaaggctattggtcaaggc

SEQ ID NO: 42 - DNA, 83 bp, Artificial Sequence
  ssODN_3
cctagccagccgccggcccctggcctcactggatactctatcttattggtcaagtttgccttgtcaaggctattggtcaaggc

SEQ ID NO: 43 - DNA, 83 bp, Artificial Sequence
  ssODN_4
cctagccagccgccggcccctggcctcactggatactctatcatattggtcaagtttgccttgtcaaggctattggtcaaggc

SEQ ID NO: 44 - DNA, 82 bp, Artificial Sequence
  ssODN_5
ctctaagactattggtcaagtttgccttgtcaaggctatctgtcaaggcaaggctggccaacccatgggtggagtttagcca

SEQ ID NO: 45 - DNA, 82 bp, Artificial Sequence
  ssODN_6
ctctaagactattggtcaagtttgccttgtcaaggctatcagtcaaggcaaggctggccaacccatgggtggagtttagcca

SEQ ID NO: 46 - DNA, 82 bp, Artificial Sequence
  ssODN_7
ctctaagactattggtcaagtttgccttgtcaaggctatctctcaaggcaaggctggccaacccatgggtggagtttagcca

SEQ ID NO: 47 - DNA, 82 bp, Artificial Sequence
  ssODN_8
ctctaagactattggtcaagtttgccttgtcaaggctatcactcaaggcaaggctggccaacccatgggtggagtttagcca

SEQ ID NO: 48 - DNA, 82 bp, Artificial Sequence
  ssODN_9
ctctaagactattggtcaagtttgccttgtcaaggctatctttcaaggcaaggctggccaacccatgggtggagtttagcca

SEQ ID NO: 49 - DNA, 82 bp, Artificial Sequence
  ssODN_10
ctctaagactattggtcaagtttgccttgtcaaggctatcattcaaggcaaggctggccaacccatgggtggagtttagcca

SEQ ID NO: 50 - DNA, 82 bp, Artificial Sequence
  ssODN_11
ctctaagactattggtcaagtttgccttgtcaaggctatctatcaaggcaaggctggccaacccatgggtggagtttagcca

SEQ ID NO: 51 - DNA, 82 bp, Artificial Sequence
  ssODN_12
ctctaagactattggtcaagtttgccttgtcaaggctatcaatcaaggcaaggctggccaacccatgggtggagtttagcca

SEQ ID NO: 52 - DNA, 82 bp, Artificial Sequence
  ssODN_13
ctctaagactattggtcaagtttgccttgtcaaggctatttatcaaggcaaggctggccaacccatgggtggagtttagcca

SEQ ID NO: 53 - DNA, 83 bp, Artificial Sequence
  ssODN_14
ctctaagactattggtcaagtttgccttgtcaaggctattttatcaaggcaaggctggccaacccatgggtggagtttagcca

SEQ ID NO: 54 - DNA, 81 bp, Artificial Sequence
  ssODN_15
ctctaagactattggtcaagtttgccttgtcaaggctattatcaaggcaaggctggccaacccatgggtggagtttagcca

SEQ ID NO: 55 - DNA, 78 bp, Artificial Sequence
  ssODN_16
ctctaagactattggtcaagtttgccttgtcaaggctatcaaggcaaggctggccaacccatgggtggagtttagcca

SEQ ID NO: 56 - DNA, 81 bp, Artificial Sequence
  ssODN_17
cctcactggatactctaagactattggtcaagtttgccttatcaaggcaaggctggccaacccatgggtggagtttagcca

SEQ ID NO: 57 - DNA, 82 bp, Artificial Sequence
  ssODN_18
cctcactggatactctaagactattggtcaagtttgcctttatcaaggcaaggctggccaacccatgggtggagtttagcca

SEQ ID NO: 58 - DNA, 81 bp, Artificial Sequence
  ssODN_19
tggctaaactccacccatgggttggccagccttgccttgataaggcaaacttgaccaatagtcttagagtatccagtgagg

SEQ ID NO: 59 - DNA, 82 bp, Artificial Sequence
  ssODN_20
tggctaaactccacccatgggttggccagccttgccttgataaaggcaaacttgaccaatagtcttagagtatccagtgagg

SEQ ID NO: 60 - DNA, 86 bp, Artificial Sequence
  ssODN_21
tccccacactatctcaatgcaaatatctgtctgaaacggtagataaccctggctaaactccacccatgggttggccagccttgcct

SEQ ID NO: 61 - DNA, 84 bp, Artificial Sequence
  ssODN_22
tatcctcttgggggccccttccccacactatctcaatgcaacagaaacggtccctggctaaactccacccatgggttggccagc

SEQ ID NO: 62 - DNA, 83 bp, Artificial Sequence
  ssODN_23
cctatgcctaaaacacatttcacaatccctgaacttttcagataattggtacatgctttaactttaaactacaggcctcactg

SEQ ID NO: 63 - DNA, 84 bp, Artificial Sequence
  ssODN_24
cctatgcctaaaacacatttcacaatccctgaacttttcagataaattggtacatgctttaactttaaactacaggcctcactg

SEQ ID NO: 64 - DNA, 85 bp, Artificial Sequence
  ssODN_25
cctatgcctaaaacacatttcacaatccctgaacttttcagataaaattggtacatgctttaactttaaactacaggcctcactg

SEQ ID NO: 65 - DNA, 85 bp, Artificial Sequence
  ssODN_26
cctatgcctaaaacacatttcacaatccctgaacttttcagatagaattggtacatgctttaactttaaactacaggcctcactg

SEQ ID NO: 66 - RNA, 80 nt, Artificial Sequence
  synthetic
guuuuagagcuagaaauagcaaguuaaaauaaggcuaguccguuaucaacuugaaaaaguggcaccgagucggugcuuuu

SEQ ID NO: 67 - DNA, 24 bp, Artificial Sequence
  synthetic
ggactatcatatgcttaccgtaac

SEQ ID NO: 68 - DNA, 20 bp, Artificial Sequence
  synthetic
ggcgggccatttaccgtaag

SEQ ID NO: 69 - RNA, 100 nt, Artificial Sequence
  sgRNA-1
acuggauacucuaagacuauguuuuagagcuagaaauagcaaguuaaaauaaggcuaguccguuaucaacuugaaaaaguggcaccgagucggugcuuuu

SEQ ID NO: 70 - RNA, 100 nt, Artificial Sequence
  sgRNA-2
cuugucaaggcuauuggucaguuuuagagcuagaaauagcaaguuaaaauaaggcuaguccguuaucaacuugaaaaaguggcaccgagucggugcuuuu

SEQ ID NO: 71 - RNA, 100 nt, Artificial Sequence
  sgRNA-3
guuugccuugucaaggcuauguuuuagagcuagaaauagcaaguuaaaauaaggcuaguccguuaucaacuugaaaaaguggcaccgagucggugcuuuu

SEQ ID NO: 72 - RNA, 100 nt, Artificial Sequence
  sgRNA-4
uggucaaguuugccuugucaguuuuagagcuagaaauagcaaguuaaaauaaggcuaguccguuaucaacuugaaaaaguggcaccgagucggugcuuuu

SEQ ID NO: 73 - RNA, 100 nt, Artificial Sequence
  sgRNA-5
cuugaccaauagccuugacaguuuuagagcuagaaauagcaaguuaaaauaaggcuaguccguuaucaacuugaaaaaguggcaccgagucggugcuuuu

SEQ ID NO: 74 - RNA, 100 nt, Artificial Sequence
  sgRNA-6
uaucugucugaaacggucccguuuuagagcuagaaauagcaaguuaaaauaaggcuaguccguuaucaacuugaaaaaguggcaccgagucggugcuuuu

SEQ ID NO: 75 - RNA, 100 nt, Artificial Sequence
  sgRNA-7
augcaaauaucugucugaaaguuuuagagcuagaaauagcaaguuaaaauaaggcuaguccguuaucaacuugaaaaaguggcaccgagucggugcuuuu

SEQ ID NO: 76 - RNA, 100 nt, Artificial Sequence
  sgRNA-8
ucccugaacuuuucaaaaauguuuuagagcuagaaauagcaaguuaaaauaaggcuaguccguuaucaacuugaaaaaguggcaccgagucggugcuuuu

SEQ ID NO: 77 - DNA, 22 bp, Homo sapiens
tactgcgctgaaactgtggctt

SEQ ID NO: 78 - DNA, 22 bp, Homo sapiens
cttcccagggtttctcctccag

SEQ ID NO: 79 - DNA, 26 bp, Homo sapiens
tgcactgaaactgttgctttatagga